European Patent Application EP 4 283 296 A1, published November 29, 2023. Title: VIRUS-LIKE PARTICLES COMPRISING TOXOPLASMA PROTEIN AND INFLUENZA PROTEIN AND DIAGNOSTIC METHOD USING THE SAME. Applicant: health park co,.ltd. The sequence listing filed with the application follows.

SEQUENCE LISTING (16 sequences)

SEQ ID NO: 1 - protein, 252 aa, Artificial Sequence
  Influenza virus matrix protein 1(M1) Amino acid sequence
MSLLTEVETYVLSIIPSGPLKAEIAQRLEDVFAGKNTDLEVLMEWLKTRPILSPLTKGILGFVFTLTVPSERGLQRRRFVQNALNGNGDPNNMDKAVKLYRKLKREITFHGAKEISLSYSAGALASCMGLIYNRMGAVTTEVAFGLVCATCEQIADSQHRSHRQMVTTTNPLIRHENRMVLASTTAKAMEQMAGSSEQAAEAMEVASQARQMVQAMRTIGTHPSSSAGLKNDLLENLQAYQKRMGVQMQRFK

SEQ ID NO: 2 - protein, 541 aa, Artificial Sequence
  TgAMA1 Amino acid sequence
MGLVGVQVLLVLVADCTIFASGLSSSTRSRESQTLSASTSGNPFQANVEMKTFMERFNLTHHHQSGIYVDLGQDKEVDGTLYREPAGLCPIWGKHIELQQPDRLPYRNNFLEDVPTEKEYKQSGNPLPGGFNLNFVTPSGQRISPFPMELLEKNSNIKASTDLGRCAEFAFKTVAMDKNNKATKYRYPFVYDSKKRLCHILYVSMQLMEGKKYCSVKGEPPDLTWYCFKPRKSVTENHHLIYGSAYVGENPDAFISKCPNQALRGYRFGVWKKGRCLDYTELTDTVIERVESKAQCWVKTFENDGVASDQPHTYPLTSQASWNDWWPLHQSDQPHSGGVGRNYGFYYVDTTGEGKCALSDQVPDCLVSDSAAVSYTAAGSLSEETPNFIIPSNPSVTPPTPETALQCTADKFPDSFGACDVQACKRQKTSCVGGQIQSTSVDCTADEQNECGSNTALIAGLAVGGVLLLALLGGGCYFAKRLDRNKGVQAAHHEHEFQSDRGARKKRPSDLMQEAEPSFWDEAEENIEQDGETHVMVEGDY

SEQ ID NO: 3 - protein, 578 aa, Artificial Sequence
  TgROP4 Amino acid sequence
MGHPTSFGQPSCLVWLAAAFLVLGLCLVQQGAGRQRPHQWKSSEAALSVSPAGDIVDKYSRDSTEGENTVSEGEAEGSRGGSWLEQEGVELRSPSQDSQTGTSTASPTGFRRLLRRLRFWRRGSTRGSDDAAEVSRRTRVPLHTRLLQHLRRVARIIRHGVSAAAGRLFGRVRQVEAERPQPVFTEGDPPDLETNSLYYRDKVPGQGIIQEILRQKPGIAHHPESFSVVAADERVSRTLWAEGGVVRVASELGQPGRVLVRGRRIGLFRPGMQFEATDQATGEPMTALVGHTVLEATARDVDSMRNEGLAVGLFQKVKNPYLANRYLRFLAPFDLVTIPGKPLVQKAKSRNEVGWVKNLLFLLPPTHVDMETFVDEIGRFPQEDRPLADAARLYLTVQAVRLVAHLQDEGVVHGKIMPDSFCLKREGGLYLRDFGSLVRAGAKVVVPAEYDEYTPPEGRAAARSRFGSGATTMTYAFDAWTLGSVIFLIWCSRAPDTKSGYEYSVEFFFSRCRRVPENVKLLVYKLINPSVEARLLALQAIETPEYREMEEQLSAASRLYSGDGTLTGGDDDMPPLET

SEQ ID NO: 4 - protein, 554 aa, Artificial Sequence
  TgROP18 Amino acid sequence
MFSVQRPPLTRTVVRMGLATLLPKTACLAGLNVALVFLLFQVQDGTGITLGPSKLDSKPTSLDSQQHVADKRWLATVGHYKHLAGATESTRDVSLLEERAQHRVNAQETNQRRTIFQRLLNLLRRRERDGEVSGSAADSSSRPRLSVRQRLAQLWRRAKSLFKRGIRRYFPQGRNRQRSLRAQRRRSELVFEKADSGCVIGKRILAHMQEQIGQPQALENSERLDRILTVAAWPPDVPKRFVSVTTGETRTLVRGAPLGSGGFATVYEATDVETNEELAVKVFMSEKEPTDETMLDLQRESSCYRNFSLAKTAKDAQESCRFMVPSDVVMLEGQPASTEVVIGLTTRWVPNYFLLMMRAEADMSKVISWVFGDASVNKSEFGLVVRMYLSSQAIKLVANVQAQGIVHTDIKPANFLLLKDGRLFLGDFGTYRINNSVGRAIGTPGYEPPERPFQATGITYTFPTDAWQLGITLYCIWCKERPTPADGIWDYLHFADCPSTPELVQDLIRSLLNRDPQKRMLPLQALETAAFKEMDSVVKGAAQNFEQQEHLHTE

SEQ ID NO: 5 - DNA, 1027 bp, Artificial Sequence
  Influenza virus matrix protein 1(M1) DNA sequence
agcgaaagcaggtagatattgaaagatgagtcttctaaccgaggtcgaaacgtacgtactctctatcatcccgtcaggccccctcaaagccgagatcgcacagagacttgaagatgtctttgcagggaagaacaccgatcttgaggttctcatggaatggctaaagacaagaccaatcctgtcacctctgactaaggggattttaggatttgtgttcacgctcaccgtgcccagtgagcgaggactgcagcgtagacgctttgtccaaaatgcccttaatgggaacggggatccaaataacatggacaaagcagttaaactgtataggaagctcaagagggagataacattccatggggccaaagaaatctcactcagttattctgctggtgcacttgccagttgtatgggcctcatatacaacaggatgggggctgtgaccactgaagtggcatttggcctggtatgtgcaacctgtgaacagattgctgactcccagcatcggtctcataggcaaatggtgacaacaaccaatccactaatcagacatgagaacagaatggttttagccagcactacagctaaggctatggagcaaatggctggatcgagtgagcaagcagcagaggccatggaggttgctagtcaggctagacaaatggtgcaagcgatgagaaccattggaactcatcctagctccagtgctggtctgaaaaatgatcttcttgaaaatttgcaggcctatcagaaacgaatgggggtgcagatgcaacggttcaagtgatcctctcactattgccgcaaatatcattgggatcttgcacttgacattgtggattcttgatcgtctttttttcaaatgcatttaccgtcgctttaaatacggactgaaaggagggccttctacggaaggagtgccaaagtctatgagggaagaatatcgaaaggaacagcagagtgctgtggatgctgacgatggtcattttgtcagcatagagctggagtaaaaaactaccttgtttctact

SEQ ID NO: 6 - DNA, 1626 bp, Artificial Sequence
  TgAMA1 DNA sequence
atggggctcgtgggcgtacaagttttgctggttcttgtggcggattgcaccatattcgcatcgggactcagctcaagcacaaggtctcgcgagtcgcagacgctgagtgctagcacgtcggggaatccctttcaggcaaatgtagagatgaaaaccttcatggaaagattcaacctaactcatcatcatcagtctggtatttacgtcgaccttggacaagacaaggaagttgatggcacattataccgggagcctgcggggttgtgtcccatttggggaaagcacatcgaactccagcagccggaccggcttccgtaccgtaacaacttcttggaagatgttccgactgaaaaagaatacaaacagtcagggaatcctttgcccggaggcttcaacttgaatttcgtgacgcctagcgggcagcgaatttcaccatttccgatggaacttcttgaaaaaaatagcaacatcaaggcgagtacggatcttgggaggtgcgccgagtttgcctttaagacggtcgctatggataaaaacaataaggcgacgaagtaccgttacccatttgtttatgactccaagaagcgactgtgccacatcctctacgtatcgatgcagctgatggagggtaaaaagtactgttcagtcaagggcgaacctccagatctcacatggtattgcttcaagccccgaaagagtgttacggagaatcatcatctcatctacggatcggcctatgttggagagaacccagatgcgttcatcagtaaatgcccaaatcaagctcttcgcgggtacaggttcggtgtttggaagaaaggccgttgcctcgactacactgaattgaccgacactgtgatagaacgtgttgagtcaaaggcacagtgctgggtgaaaacctttgaaaacgacggggtcgcgagtgaccaaccccatacgtatccactgacgtcgcaagcatcatggaacgattggtggcctctccaccagagtgaccaacctcactcaggtggcgttgggcgtaattacggtttctactacgtggacacgactggagagggcaagtgtgcactctctgaccaggtacccgactgcctggtgtcggattctgccgccgtgtcgtatacagcagcggggagtttgtctgaagagacgccgaatttcataattccgtcaaatccctctgttactccgccaacgcccgagacggcacttcagtgcacggccgacaagttccccgactctttcggtgcctgcgacgttcaagcctgtaaaagacagaagacgtcctgcgttggcggacagattcaaagtactagcgtcgactgcaccgcggacgaacaaaatgaatgtggctctaacactgcgttgatcgctggactcgccgtaggaggggttctgctgttggctcttctaggaggaggctgctacttcgcgaagaggttggacagaaacaaaggcgtccaggcggctcatcatgaacatgagtttcagtcagacagaggtgctcgaaaaaagaggccaagcgatctcatgcaagaggctgaaccgtcgttttgggatgaggcagaggagaacattgaacaagatggggaaacacatgttatggtcgagggggattactag

SEQ ID NO: 7 - DNA, 2039 bp, Artificial Sequence
  TgROP4 DNA sequence
tccggcatggaaaaaatgcgtctagctaaccgcgggccccaatgtcgcacggccttggtcaagggacggcgcgacctgcagagacgggaatccgagccaagcgctgagtgtccttgcttctggctgagccgccatcctgcggcaccgtccatgactgcgcacagcatcccgggagtatggtgattgtgtcagtcttatttcttttgaaggcacttcagatgtgtacttcagaatgttgttacgataattgcggatgcagctgccacctctgaacggttgatttggttgtgagtcctcccaacatggggcaccctacctctttcggacagccgtcgtgtcttgtctggctagctgcggcattccttgttctggggctttgcctcgtccagcaaggcgctggcagacagcggcctcaccagtggaagagctcggaagccgctttgagtgtcagtccggcaggagacatcgtggacaagtattctcgtgattccactgagggagaaaacactgtctcagagggggaagctgagggcagtcgggggggttcatggctggagcaggagggggttgaattaaggtcgccttcacaggacagccagacaggaacctcgaccgcgtcccccacaggcttcagaaggttactcaggcgtttgcgtttttggcgtcgtgggagtacacgcggatccgatgatgcagcagaagtttccaggaggactcgggttcctctgcatacccgtctgcttcagcatttgcggcgagtagcgagaatcatccgacacggggtttcagcggccgctggcagattgttcgggcgagttcggcaagttgaggcggaacgtccacaacccgttttcactgaaggtgatcctccggatctcgagacgaattccttgtattatcgcgacaaggttccaggacaggggataatccaggagatcctcaggcagaagccgggaatcgcacaccaccccgagtcatttagtgtggttgctgctgacgagagagtatcacggactctgtgggctgagggcggggttgtgagagttgcttcagaattgggccaacctgggagagtgctcgtgagggggagacgaatcggtttgtttcgcccaggaatgcagtttgaagcaacagaccaggcgacaggagaaccgatgactgcgcttgttggccatactgtgcttgaggccacggcaagagacgtagattcgatgcgcaacgaaggattagctgttgggttgtttcaaaaggtgaagaacccatatctagctaacaggtatctaagatttctggccccgttcgatttggtgacgatcccggggaagccattagttcagaaagctaagtcacgtaatgaggttggctgggtcaaaaatctgttgtttctgcttcctccaactcatgtcgatatggaaacgtttgtcgacgagattggtcgatttccacaagaggaccgccccctagctgatgccgctcgattgtatcttactgttcaggcggtgaggttggtagcgcacctccaagacgaaggagtggtgcacgggaagataatgcctgattcgttttgtttgaagcgtgaggggggcctgtacttgcgtgactttggctctctggtgagagcgggcgcaaaagtggtggtgcccgcggaatatgatgagtatacgccgccagaaggtcgtgcggccgcccgaagtcgtttcggctctggggcgaccacgatgacgtacgcattcgacgcctggacactgggttcggttatatttttaatttggtgctctcgagctcccgatacaaaatcggggtacgaatacagtgtcgaattctttttttcgaggtgccggcgggtgccagagaacgtgaaacttctggtttacaagttgattaacccttctgtcgaggcccgcctgctcgccttgcaagcgatagagactccggaatacagggagatggaagaacagctgtccgctgcttcgcgcctgtactcaggtgatgggacgttgacagggggagacgatgacatgccaccactggaaacgtga

SEQ ID NO: 8 - DNA, 1665 bp, Artificial Sequence
  TgROP18 DNA sequence
atgttttcggtacagcggccacctcttacgcgtaccgtcgtccgaatgggtttagcgactcttctcccgaagacagcctgtcttgcggggttaaatgtagcgcttgtcttcctgctcttccaagtccaggatgggaccggaatcacacttggtccttcaaaactcgactccaaaccgacaagtttggattcgcaacagcacgttgctgacaagcggtggcttgctacagttggccactacaaacatttagcaggagcgacagaaagcactcgagacgtttcattgctggaggaaagggctcaacaccgggtaaatgcgcaagaaacaaaccaacggcgcacgatttttcagaggcttctgaatctcttgagacggagagaaagagatggtgaagtctcgggttccgcagctgatagctcctcgagaccccgtctgtccgtacgacagaggcttgctcaactttggcgtagagcgaaatcgttattcaaacgcggaatccggaggtactttcctcaagggcgtaaccgacagcgaagtttgcgggcacaaagacggcgatctgaattggtttttgagaaggcggattctggatgcgtcatcggcaaacgcatcctggcgcacatgcaagaacaaatcgggcagcctcaagcgctagaaaatagtgaacgactggatagaattctgactgtcgccgcctggcctccggacgttccaaaaagatttgtttctgtgactaccggtgaaacccggacgctggtgagaggtgcaccccttggctctggtggattcgccactgtatatgaggctacagacgtggagacgaatgaagagttggctgttaaggttttcatgtcagaaaaggagcccaccgatgagactatgcttgacttgcagagggagtcgtcctgctacaggaactttagtctagccaagacggcgaaggatgcccaggaaagctgtagattcatggttcctagtgatgttgtgatgttagagggacagccagcatccacagaggtcgtgattggtttgacgactcggtgggtaccaaactattttcttctcatgatgcgggcagaagcggacatgagcaaagtcatttcatgggtatttggagatgcgtctgtcaataaaagtgaatttggcctggtcgttcgaatgtacctatccagtcaggcaatcaaactagtggccaatgttcaagctcagggaattgtgcatacggatatcaaaccggcgaatttcctcctcttgaaagacggtcgcctgtttctcggcgacttcggaacgtatagaatcaataattcggttggacgcgcgataggtactcccggttacgagcctccggagcgaccgtttcaggctacaggcatcacctatacattccccactgacgcgtggcaactcggtataactttgtactgcatctggtgcaaggaacgtccaactccggccgacggcatctgggactacttacacttcgcagattgtccttccacgcctgagctggttcaagacctcatccgaagcctcttgaatcgagatcctcagaaacggatgctcccgctacaagccttggagacagcagcgtttaaagagatggattcagtagtaaaaggcgccgcgcaaaacttcgaacagcaggaacatctccacacagaataa

SEQ ID NO: 9 - DNA, 32 bp, Artificial Sequence
  M1 primer F
aaaggatccaccatgagtcttctaaccgaggt

SEQ ID NO: 10 - DNA, 30 bp, Artificial Sequence
  M1 primer R
ttactcgagttactctagctctatgttgac

SEQ ID NO: 11 - DNA, 32 bp, Artificial Sequence
  AMA1 primer F
aaagaattcaccatggggctcgtgggcgtaca

SEQ ID NO: 12 - DNA, 29 bp, Artificial Sequence
  AMA1 primer R
ttactcgagctagtaatccccctcgacca

SEQ ID NO: 13 - DNA, 32 bp, Artificial Sequence
  ROP4 primer F
aaagcatgcaccatggggcaccctacctcttt

SEQ ID NO: 14 - DNA, 30 bp, Artificial Sequence
  ROP4 primer R
ttaggtacctcacgtttccggtggtggcat

SEQ ID NO: 15 - DNA, 32 bp, Artificial Sequence
  ROP18 primer F
aaaggatccaccatgttttcggtacagcggcc

SEQ ID NO: 16 - DNA, 30 bp, Artificial Sequence
  ROP18 primer R
ttatctagattattctgtgtggagatgttc